European Patent Specification EP 3 922 646 B1, published November 26, 2025. Title: ANTIBODIES FOR TREATING MALIGNANT TUMORS AND USES THEREOF. Applicant: SHENZHEN UNIVERSITY. The sequence listing filed with the application follows.

SEQUENCE LISTING (8 sequences)

SEQ ID NO: 1 - protein, 106 aa, Artificial Sequence
DIVLTQSPAIMSASPGEKVTMTCSASSSVTYTYWYQQKPGSSPRLLIYDTSNLASGVPVRFSGSGSGTSYSLTISRMEAEDAATYYCQQWSSYPFTFGSGTKLEIK

SEQ ID NO: 2 - protein, 120 aa, Artificial Sequence
QLQLQQSGPELVKPGASVRMSCKAAGYTFTSYLMHWVKQRPGQDLEWIGYINPYNDGTKYNEKFKDKATLTSDKSSSTVYMELSSLTSEDSAVYYCARSDVYYGVRFAYWGQGTLVTVSA

SEQ ID NO: 3 - protein, 213 aa, Artificial Sequence
DIVLTQSPAIMSASPGEKVTMTCSASSSVTYTYWYQQKPGSSPRLLIYDTSNLASGVPVRFSGSGSGTSYSLTISRMEAEDAATYYCQQWSSYPFTFGSGTKLEIKRTVAAPSVFIFPPSDEQLKSGTASVVCLLNNFYPREAKVQWKVDNALQSGNSQESVTEQDSKDSTYSLSSTLTLSKADYEKHKVYACEVTHQGLSSPVTKSFNRGEC

SEQ ID NO: 4 - protein, 450 aa, Artificial Sequence
QLQLQQSGPELVKPGASVRMSCKAAGYTFTSYLMHWVKQRPGQDLEWIGYINPYNDGTKYNEKFKDKATLTSDKSSSTVYMELSSLTSEDSAVYYCARSDVYYGVRFAYWGQGTLVTVSAASTKGPSVFPLAPSSKSTSGGTAALGCLVKDYFPEPVTVSWNSGALTSGVHTFPAVLQSSGLYSLSSVVTVPSSSLGTQTYICNVNHKPSNTKVDKKVEPKSCDKTHTCPPCPAPELLGGPSVFLFPPKPKDTLMISRTPEVTCVVVDVSHEDPEVKFNWYVDGVEVHNAKTKPREEQYNSTYRVVSVLTVLHQDWLNGKEYKCKVSNKALPAPIEKTISKAKGQPREPQVYTLPPSRDELTKNQVSLTCLVKGFYPSDIAVEWESNGQPENNYKTTPPVLDSDGSFFLYSKLTVDKSRWQQGNVFSCSVMHEALHNHYTQKSLSLSPGK

SEQ ID NO: 5 - protein, 318 aa, Artificial Sequence
GACATCGTGCTGACCCAGTCTCCAGCCATCATGTCTGCTAGCCCTGGCGAGAAAGTGACAATGACCTGCTCCGCCTCCTCCTCCGTGACCTACACCTACTGGTATCAGCAGAAGCCCGGCTCCAGTCCTCGGCTGCTGATCTACGATACCTCCAACCTGGCTTCTGGCGTGCCCGTGCGGTTTTCTGGTTCTGGCTCTGGCACCTCCTACAGCCTGACCATCTCCAGAATGGAAGCCGAGGATGCCGCCACCTACTACTGTCAGCAGTGGTCTAGCTACCCCTTCACCTTTGGCTCCGGCACCAAGCTGGAAATCAAG

SEQ ID NO: 6 - protein, 360 aa, Artificial Sequence
CAGTTGCAGCTCCAGCAGTCTGGACCTGAGCTGGTTAAGCCTGGTGCCTCCGTCCGGATGTCTTGCAAGGCTGCCGGCTACACCTTCACCAGCTACCTGATGCACTGGGTCAAGCAGAGGCCAGGCCAGGACTTGGAGTGGATCGGCTACATCAACCCCTACAACGACGGCACCAAGTACAACGAGAAGTTCAAGGACAAGGCTACCCTGACCTCCGACAAGTCCTCCTCCACCGTGTACATGGAACTGTCCAGCCTGACCTCTGAGGACTCCGCCGTGTACTACTGCGCCAGATCCGATGTGTACTATGGCGTCAGATTCGCCTACTGGGGCCAGGGCACACTGGTCACAGTTTCTGCT

SEQ ID NO: 7 - protein, 639 aa, Artificial Sequence
GACATCGTGCTGACCCAGTCTCCAGCCATCATGTCTGCTAGCCCTGGCGAGAAAGTGACAATGACCTGCTCCGCCTCCTCCTCCGTGACCTACACCTACTGGTATCAGCAGAAGCCCGGCTCCAGTCCTCGGCTGCTGATCTACGATACCTCCAACCTGGCTTCTGGCGTGCCCGTGCGGTTTTCTGGTTCTGGCTCTGGCACCTCCTACAGCCTGACCATCTCCAGAATGGAAGCCGAGGATGCCGCCACCTACTACTGTCAGCAGTGGTCTAGCTACCCCTTCACCTTTGGCTCCGGCACCAAGCTGGAAATCAAGAGAACAGTGGCCGCTCCTAGCGTGTTCATCTTCCCACCTTCCGACGAGCAGCTGAAGTCTGGCACAGCCTCTGTCGTGTGCCTGCTGAACAACTTCTACCCCAGAGAAGCCAAGGTGCAGTGGAAGGTGGACAACGCCCTGCAGAGCGGCAATAGCCAAGAGAGCGTGACCGAGCAGGACAGCAAGGACTCTACCTACAGCCTGAGCAGCACCCTGACACTGAGCAAGGCCGACTACGAGAAGCACAAAGTGTACGCCTGCGAAGTGACCCACCAGGGCCTTTCTAGCCCTGTGACCAAGAGCTTCAACCGGGGCGAATGT

SEQ ID NO: 8 - protein, 1350 aa, Artificial Sequence
CAGTTGCAGCTCCAGCAGTCTGGACCTGAGCTGGTTAAGCCTGGTGCCTCCGTCCGGATGTCTTGCAAGGCTGCCGGCTACACCTTCACCAGCTACCTGATGCACTGGGTCAAGCAGAGGCCAGGCCAGGACTTGGAGTGGATCGGCTACATCAACCCCTACAACGACGGCACCAAGTACAACGAGAAGTTCAAGGACAAGGCTACCCTGACCTCCGACAAGTCCTCCTCCACCGTGTACATGGAACTGTCCAGCCTGACCTCTGAGGACTCCGCCGTGTACTACTGCGCCAGATCCGATGTGTACTATGGCGTCAGATTCGCCTACTGGGGCCAGGGCACACTGGTCACAGTTTCTGCTGCCTCTACAAAGGGCCCTAGTGTGTTCCCTCTGGCTCCCAGCAGCAAGTCTACATCTGGCGGAACAGCCGCTCTGGGCTGCCTGGTCAAGGATTACTTTCCCGAGCCTGTGACCGTGTCCTGGAATAGCGGAGCACTGACAAGCGGCGTGCACACCTTTCCAGCTGTGCTGCAAAGCAGCGGCCTGTACTCTCTGAGCAGCGTGGTCACAGTGCCTAGCTCTAGCCTGGGCACCCAGACCTACATCTGCAATGTGAACCACAAGCCTAGCAACACCAAGGTGGACAAGAAGGTGGAACCCAAGAGCTGCGACAAGACCCACACCTGTCCTCCATGTCCTGCTCCAGAACTGCTCGGCGGACCTTCCGTGTTCCTGTTTCCTCCAAAGCCTAAGGACACCCTGATGATCAGCAGAACCCCTGAAGTGACCTGCGTGGTGGTGGATGTGTCCCACGAGGATCCCGAAGTGAAGTTCAATTGGTACGTGGACGGCGTGGAAGTGCACAACGCCAAGACCAAGCCTAGAGAGGAACAGTACAACAGCACCTACAGAGTGGTGTCCGTGCTGACCGTGCTGCACCAGGATTGGCTGAACGGCAAAGAGTACAAGTGCAAGGTGTCCAACAAGGCCCTGCCTGCTCCTATCGAGAAAACCATCAGCAAGGCCAAGGGCCAGCCTAGGGAACCCCAGGTTTACACACTGCCTCCAAGCAGGGACGAGCTGACCAAGAATCAGGTGTCCCTGACCTGCCTCGTGAAGGGCTTCTACCCTTCCGATATCGCCGTGGAATGGGAGAGCAATGGCCAGCCTGAGAACAACTACAAGACAACCCCTCCTGTGCTGGACAGCGACGGCTCATTCTTCCTGTACAGCAAGCTGACAGTGGACAAGTCCAGATGGCAGCAGGGCAACGTGTTCAGCTGCAGCGTGATGCACGAGGCCCTGCACAACCACTACACCCAGAAGTCCCTGAGCCTGTCTCCTGGCAAA